European Patent Application EP 4 342 492 A1, published March 27, 2024. Title: PHARMACEUTICAL COMBINATION AND USE THEREOF. Applicant: TIANJIN LIPOGEN TECHNOLOGY CO.,LTD. The sequence listing filed with the application follows.

SEQUENCE LISTING (44 sequences)

SEQ ID NO: 1 - protein, 8 aa, Artificial Sequence
  RB00004 HCDR1
GFTFSSYT

SEQ ID NO: 2 - protein, 8 aa, Artificial Sequence
  RB00004 HCDR2
ISNGGSFT

SEQ ID NO: 3 - protein, 12 aa, Artificial Sequence
  RB00004 HCDR3
ARDSDYYGIFDY

SEQ ID NO: 4 - protein, 25 aa, Artificial Sequence
  RB00004 HFR1
EVQLVESGGGLVKPGGSLRLSCAAS

SEQ ID NO: 5 - protein, 17 aa, Artificial Sequence
  RB00004 HFR2
MSWVRQAPGKGLEWVAT

SEQ ID NO: 6 - protein, 38 aa, Artificial Sequence
  RB00004 HFR3
YYPDSMKGRFTISRDNSKNTLYLQMSSLRAEDTAVYYC

SEQ ID NO: 7 - protein, 11 aa, Artificial Sequence
  RB00004 HFR4；RB00005 HFR4；
WGQGTTVTVSS

SEQ ID NO: 8 - protein, 119 aa, Artificial Sequence
  RB00004 VH
EVQLVESGGGLVKPGGSLRLSCAASGFTFSSYTMSWVRQAPGKGLEWVATISNGGSFTYYPDSMKGRFTISRDNSKNTLYLQMSSLRAEDTAVYYCARDSDYYGIFDYWGQGTTVTVSS

SEQ ID NO: 9 - protein, 446 aa, Artificial Sequence
  RB00004 HC
EVQLVESGGGLVKPGGSLRLSCAASGFTFSSYTMSWVRQAPGKGLEWVATISNGGSFTYYPDSMKGRFTISRDNSKNTLYLQMSSLRAEDTAVYYCARDSDYYGIFDYWGQGTTVTVSSASTKGPSVFPLAPCSRSTSESTAALGCLVKDYFPEPVTVSWNSGALTSGVHTFPAVLQSSGLYSLSSVVTVPSSSLGTKTYTCNVDHKPSNTKVDKRVESKYGPPCPPCPAPEFLGGPSVFLFPPKPKDTLMISRTPEVTCVVVDVSQEDPEVQFNWYVDGVEVHNAKTKPREEQFNSTYRVVSVLTVLHQDWLNGKEYKCKVSNKGLPSSIEKTISKAKGQPREPQVYTLPPSQEEMTKNQVSLTCLVKGFYPSDIAVEWESNGQPENNYKTTPPVLDSDGSFFLYSRLTVDKSRWQEGNVFSCSVMHEALHNHYTQKSLSLSLGK

SEQ ID NO: 10 - protein, 16 aa, Artificial Sequence
  RB00004 LCDR1
RSSKSLLYKDGKTYLN

SEQ ID NO: 11 - protein, 7 aa, Artificial Sequence
  RB00004 LCDR2
LMSTRAS

SEQ ID NO: 12 - protein, 9 aa, Artificial Sequence
  RB00004 LCDR3
QQLVEDPFT

SEQ ID NO: 13 - protein, 23 aa, Artificial Sequence
  RB00004 LFR1
DIVMTQSPLSLPVTPGEPASISC

SEQ ID NO: 14 - protein, 15 aa, Artificial Sequence
  RB00004 LFR2
WYLQKPGQSPQLLIY

SEQ ID NO: 15 - protein, 32 aa, Artificial Sequence
  RB00004 LFR3
GVPDRFSGSGSGTDFTLKISRVEAEDVGVYYC

SEQ ID NO: 16 - protein, 13 aa, Artificial Sequence
  RB00004 LFR4
FGQGTKLEIKRTV

SEQ ID NO: 17 - protein, 115 aa, Artificial Sequence
  RB00004 VL
DIVMTQSPLSLPVTPGEPASISCRSSKSLLYKDGKTYLNWYLQKPGQSPQLLIYLMSTRASGVPDRFSGSGSGTDFTLKISRVEAEDVGVYYCQQLVEDPFTFGQGTKLEIKRTV

SEQ ID NO: 18 - protein, 230 aa, Artificial Sequence
  RB00004 LC
IALSLALVTNSDIVMTQSPLSLPVTPGEPASISCRSSKSLLYKDGKTYLNWYLQKPGQSPQLLIYLMSTRASGVPDRFSGSGSGTDFTLKISRVEAEDVGVYYCQQLVEDPFTFGQGTKLEIKRTVAAPSVFIFPPSDEQLKSGTASVVCLLNNFYPREAKVQWKVDNALQSGNSQESVTEQDSKDSTYSLSSTLTLSKADYEKHKVYACEVTHQGLSSPVTKSFNRGEC

SEQ ID NO: 19 - protein, 5 aa, Artificial Sequence
  RB00005 HCDR1
KYIIH

SEQ ID NO: 20 - protein, 17 aa, Artificial Sequence
  RB00005 HCDR2
WFYPGSGNIRYNEKIKG

SEQ ID NO: 21 - protein, 12 aa, Artificial Sequence
  RB00005 HCDR3
HGELGGGYFFDY

SEQ ID NO: 22 - protein, 30 aa, Artificial Sequence
  RB00005 HFR1
EVQLVQSGAEVKKPGASVKVSCKASGYTFT

SEQ ID NO: 23 - protein, 14 aa, Artificial Sequence
  RB00005 HFR2
WVRQAPGQGLEWMG

SEQ ID NO: 24 - protein, 32 aa, Artificial Sequence
  RB00005 HFR3
RVTMTRDTSTSTVYMELSSLRSEDTAVYYCAR

SEQ ID NO: 25 - protein, 121 aa, Artificial Sequence
  RB00005 VH
EVQLVQSGAEVKKPGASVKVSCKASGYTFTKYIIHWVRQAPGQGLEWMGWFYPGSGNIRYNEKIKGRVTMTRDTSTSTVYMELSSLRSEDTAVYYCARHGELGGGYFFDYWGQGTTVTVSS

SEQ ID NO: 26 - protein, 451 aa, Artificial Sequence
  RB00005 HC
EVQLVQSGAEVKKPGASVKVSCKASGYTFTKYIIHWVRQAPGQGLEWMGWFYPGSGNIRYNEKIKGRVTMTRDTSTSTVYMELSSLRSEDTAVYYCARHGELGGGYFFDYWGQGTTVTVSSASTKGPSVFPLAPSSKSTSGGTAALGCLVKDYFPEPVTVSWNSGALTSGVHTFPAVLQSSGLYSLSSVVTVPSSSLGTQTYICNVNHKPSNTKVDKKVEPKSCDKTHTCPPCPAPELLGGPSVFLFPPKPKDTLMISRTPEVTCVVVDVSHEDPEVKFNWYVDGVEVHNAKTKPREEQYASTYRVVSVLTVLHQDWLNGKEYKCKVSNKALPAPIEKTISKAKGQPREPQVYTLPPSREEMTKNQVSLTCLVKGFYPSDIAVEWESNGQPENNYKTTPPVLDSDGSFFLYSKLTVDKSRWQQGNVFSCSVMHEALHNHYTQKSLSLSPGK

SEQ ID NO: 27 - protein, 10 aa, Artificial Sequence
  RB00005 LCDR1
  misc_feature (5)..(5): Xaa = Gly、Lys或Ser
  misc_feature (6)..(6): Xaa = Ala、Thr or Val
  misc_feature (7)..(7): Xaa = Gly or Ser
RASSXXXNIH

SEQ ID NO: 28 - protein, 10 aa, Artificial Sequence
  RB00005a LCDR1
RASSSVSNIH

SEQ ID NO: 29 - protein, 10 aa, Artificial Sequence
  RB00005b LCDR1
RASSKTGNIH

SEQ ID NO: 30 - protein, 10 aa, Artificial Sequence
  RB00005c LCDR1
RASSGASNIH

SEQ ID NO: 31 - protein, 7 aa, Artificial Sequence
  RB00005 LCDR2
ATSNLAS

SEQ ID NO: 32 - protein, 9 aa, Artificial Sequence
  RB00005 LCDR3
QQWSSNPLT

SEQ ID NO: 33 - protein, 23 aa, Artificial Sequence
  RB00005 LFR1
DIQLTQSPSFLSASVGDRVTITC

SEQ ID NO: 34 - protein, 15 aa, Artificial Sequence
  RB00005 LFR2
WYQQKPGKAPKPWIY

SEQ ID NO: 35 - protein, 32 aa, Artificial Sequence
  RB00005 LFR3
GVPSRFSGSGSGTEFTLTISSLQPEDFATYYC

SEQ ID NO: 36 - protein, 11 aa, Artificial Sequence
  RB00005 LFR4
FGQGTKLEIKR

SEQ ID NO: 37 - protein, 107 aa, Artificial Sequence
  RB00005 VL
  misc_feature (28)..(28): Xaa = Gly、Lys or Ser
  misc_feature (29)..(29): Xaa = Ala、Thr or Val
  misc_feature (30)..(30): Xaa = Gly or Ser
DIQLTQSPSFLSASVGDRVTITCRASSXXXNIHWYQQKPGKAPKPWIYATSNLASGVPSRFSGSGSGTEFTLTISSLQPEDFATYYCQQWSSNPLTFGQGTKLEIKR

SEQ ID NO: 38 - protein, 107 aa, Artificial Sequence
  RB00005a VL
DIQLTQSPSFLSASVGDRVTITCRASSSVSNIHWYQQKPGKAPKPWIYATSNLASGVPSRFSGSGSGTEFTLTISSLQPEDFATYYCQQWSSNPLTFGQGTKLEIKR

SEQ ID NO: 39 - protein, 107 aa, Artificial Sequence
  RB00005b VL
DIQLTQSPSFLSASVGDRVTITCRASSKTGNIHWYQQKPGKAPKPWIYATSNLASGVPSRFSGSGSGTEFTLTISSLQPEDFATYYCQQWSSNPLTFGQGTKLEIKR

SEQ ID NO: 40 - protein, 107 aa, Artificial Sequence
  RB00005c VL
DIQLTQSPSFLSASVGDRVTITCRASSGASNIHWYQQKPGKAPKPWIYATSNLASGVPSRFSGSGSGTEFTLTISSLQPEDFATYYCQQWSSNPLTFGQGTKLEIKR

SEQ ID NO: 41 - protein, 213 aa, Artificial Sequence
  RB00005 LC
  misc_feature (28)..(28): Xaa = Gly、Lys or Ser
  misc_feature (29)..(29): Xaa = Ala、Thr or Val
  misc_feature (30)..(30): Xaa = Gly or Ser
DIQLTQSPSFLSASVGDRVTITCRASSXXXNIHWYQQKPGKAPKPWIYATSNLASGVPSRFSGSGSGTEFTLTISSLQPEDFATYYCQQWSSNPLTFGQGTKLEIKRTVAAPSVFIFPPSDEQLKSGTASVVCLLNNFYPREAKVQWKVDNALQSGNSQESVTEQDSKDSTYSLSSTLTLSKADYEKHKVYACEVTHQGLSSPVTKSFNRGEC

SEQ ID NO: 42 - protein, 213 aa, Artificial Sequence
  RB00005a LC
DIQLTQSPSFLSASVGDRVTITCRASSSVSNIHWYQQKPGKAPKPWIYATSNLASGVPSRFSGSGSGTEFTLTISSLQPEDFATYYCQQWSSNPLTFGQGTKLEIKRTVAAPSVFIFPPSDEQLKSGTASVVCLLNNFYPREAKVQWKVDNALQSGNSQESVTEQDSKDSTYSLSSTLTLSKADYEKHKVYACEVTHQGLSSPVTKSFNRGEC

SEQ ID NO: 43 - protein, 213 aa, Artificial Sequence
  RB00005b LC
DIQLTQSPSFLSASVGDRVTITCRASSKTGNIHWYQQKPGKAPKPWIYATSNLASGVPSRFSGSGSGTEFTLTISSLQPEDFATYYCQQWSSNPLTFGQGTKLEIKRTVAAPSVFIFPPSDEQLKSGTASVVCLLNNFYPREAKVQWKVDNALQSGNSQESVTEQDSKDSTYSLSSTLTLSKADYEKHKVYACEVTHQGLSSPVTKSFNRGEC

SEQ ID NO: 44 - protein, 213 aa, Artificial Sequence
  RB00005c LC
DIQLTQSPSFLSASVGDRVTITCRASSGASNIHWYQQKPGKAPKPWIYATSNLASGVPSRFSGSGSGTEFTLTISSLQPEDFATYYCQQWSSNPLTFGQGTKLEIKRTVAAPSVFIFPPSDEQLKSGTASVVCLLNNFYPREAKVQWKVDNALQSGNSQESVTEQDSKDSTYSLSSTLTLSKADYEKHKVYACEVTHQGLSSPVTKSFNRGEC